European Patent Application EP 4 219 531 A1, published August 2, 2023. Title: Fluorescent protein sensor capable of quantitatively measuring the degree of oxidation of methionine residues of specific proteins and use thereof. Applicant: Industry Academic Cooperation Foundation of Korea University. The sequence listing filed with the application follows.

SEQUENCE LISTING (2 sequences)

SEQ ID NO: 1 - DNA, 1725 bp, Artificial Sequence
  Recombinant protein sequence for fluorescent biosensor of the present invention
aagagcaagaaaatgagtgacgaatcgaatgacgtgaagtggaacgatgccctgacaccattgcagctgatggtgctgagagataaggccactgaaaggcccaacaccggtgcgtatttacacaccaacgagtccggtgtctaccattgtgccaactgcgacagaccgttgtattcgagcaaggccaagttcgacgctcgttgtggatggcccgcattctacgaagaggtatcccctggagccatcacatatcatcgtgacaattctttaatgcctgcgagggtggagatatgttgtgcaaggtgtggtggacacttgggacatgtgtttgaaggtgaaggctggaaacagttgctaaacttgcccaaggacaccagacactgtgtgaacagtgcgtctttaaacctcaagaaggataacgtctatatcatggccgacaagcagaagaacggcatcaaggccaacttcaagatccgccacaacgtcgaggacggcagcgtgcagctcgccgaccactaccagcagaacacccccatcggcgacggccccgtgctgctgcccgacaaccactacctgagcttccagtccgtcctgagcaaagaccccaacgagaagcgcgatcacatggtcctgctggagttcgtgaccgccgccgggatcactctcggcatggacgagctgtacaacgtggatggcggtagcggtggcaccggcagcaagggcgaggagctgttcaccggggtggtgcccatcctggtcgagctggacggcgacgtaaacggccacaagttcagcgtgtccggcgagggcgagggcgatgccacctacggcaagctgaccctgaagctgatctgcaccaccggcaagctgcccgtgccctggcccaccctcgtgaccaccctcggctacggcctgaagtgcttcgcccgctaccccgaccacatgaagcagcacgacttcttcaagtccgccatgcccgaaggctacgtccaggagcgcaccatcttcttcaaggacgacggcaactacaagacccgcgccgaggtgaagttcgagggcgacaccctggtgaaccgcatcgagctgaagggcatcggcttcaaggaggacggcaacatcctggggcacaagctggagtacaacatgtcctcatacaccagtattactaaattgacgaacctaacagaatttaggaatttgatcaagcaaaatgataaactagtcatcgatttttatgctacttggtgtggcccctctaagatgatgcaaccacacttaacgaaattaattcaggcttatccagatgtaagatttgtcaagtgcgacgtggacgaatcaccagatattgccaaagagtgtgaagtgacggctatgcccacctttgttcttggcaaggatggccaactcatcggcaagatcattggagctaaccctactgctttagagaagggaatcaaagatctactggcagaggcagccgccaaggaagcggctgctaaagaagcagcagctaaagaagcggccgcgaaagcggcggctggccatggttcttctatgactacttacaaattaatccttaatggtaaaacattgaaaggcgaaacaactactgaagctgttgatgctgctactgcagaaaaagtcttcaaacaatacgctaacgacaacggtgttgacggtgaatggacttacgacgatgcgactaagacctttacagttactgaa

SEQ ID NO: 2 - protein, 575 aa, Artificial Sequence
  polynucleotide sequence encoding the recombinant protein for fluorescent biosensor of the present invention
KSKKMSDESNDVKWNDALTPLQLMVLRDKATERPNTGAYLHTNESGVYHCANCDRPLYSSKAKFDARCGWPAFYEEVSPGAITYHRDNSLMPARVEICCARCGGHLGHVFEGEGWKQLLNLPKDTRHCVNSASLNLKKDNVYIMADKQKNGIKANFKIRHNVEDGSVQLADHYQQNTPIGDGPVLLPDNHYLSFQSVLSKDPNEKRDHMVLLEFVTAAGITLGMDELYNVDGGSGGTGSKGEELFTGVVPILVELDGDVNGHKFSVSGEGEGDATYGKLTLKLICTTGKLPVPWPTLVTTLGYGLKCFARYPDHMKQHDFFKSAMPEGYVQERTIFFKDDGNYKTRAEVKFEGDTLVNRIELKGIGFKEDGNILGHKLEYNMSSYTSITKLTNLTEFRNLIKQNDKLVIDFYATWCGPSKMMQPHLTKLIQAYPDVRFVKCDVDESPDIAKECEVTAMPTFVLGKDGQLIGKIIGANPTALEKGIKDLLAEAAAKEAAAKEAAAKEAAAKAAAGHGSSMTTYKLILNGKTLKGETTTEAVDAATAEKVFKQYANDNGVDGEWTYDDATKTFTVTE